European Patent Specification EP 3 597 764 B1, published August 26, 2026. Title: MATERIALS AND METHODS FOR THE SYNTHESIS OF ERROR-MINIMIZED NUCLEIC ACID MOLECULES. Applicant: SYNTHETIC GENOMICS, INC. GIBSON, Daniel CAIAZZA, Nicky RICHARDSON, Toby. Application PCT/US2013/024496. The sequence listing filed with the application follows.

SEQUENCE LISTING (33 sequences)

SEQ ID NO: 1 - DNA, 888 bp, Selaginella lepidophylla
atggcaacgaccaagacgagcgggatggcgctggctttgctcctcgtcgccgccctggccgtgggagctgcggcctgggggaaagagggccatcgcctcacttgtatggtcgccgagccctttctaagctctgaatccaagcaagctgtggaggagcttctctctggaagagatctcccggacttgtgttcatgggccgatcagattcgaagatcgtataagtttagatggactggtcctttgcactacatcgatactccagacaacctctgcacctatgactatgatcgtgactgccacgattcccatgggaagaaggacgtgtgtgtcgctggtgggatcaacaattactcgtcgcagctggaaacgtttctagattcagagagctcgtcgtataacttgaccgaggcgctgctcttcctggctcactttgtcggggatatacaccagcccttgcacgtagcatttacgagtgatgccggaggcaatggcgtgcacgtccgctggtttggacgaaaggccaacttgcatcacgtctgggatacagaatttatttctagagccaatcgtgtgtactaccacgacatttccaagatgctccggaacattaccaggagcataactaagaagaatttcaatagttggagcagatgtaagactgatccggcggcttgtattgatagttatgcgacagaaagtatagatgcttcttgcaactgggcatacaaagacgcacccgacggaagctctctagatgatgattacttctcttcacgccttccaattgttgagcagcgtcttgctcaagggggcgtcaggctggcgtcaatactcaacaggatttttggaggagcaaagtcgaacaggtccagtcgctcaagcatgtag

SEQ ID NO: 2 - protein, 295 aa, Selaginella lepidophylla
MATTKTSGMALALLLVAALAVGAAAWGKEGHRLTCMVAEPFLSSESKQAVEELLSGRDLPDLCSWADQIRRSYKFRWTGPLHYIDTPDNLCTYDYDRDCHDSHGKKDVCVAGGINNYSSQLETFLDSESSSYNLTEALLFLAHFVGDIHQPLHVAFTSDAGGNGVHVRWFGRKANLHHVWDTEFISRANRVYYHDISKMLRNITRSITKKNFNSWSRCKTDPAACIDSYATESIDASCNWAYKDAPDGSSLDDDYFSSRLPIVEQRLAQGGVRLASILNRIFGGAKSNRSSRSSM

SEQ ID NO: 3 - DNA, 1135 bp, Apium sp.
tactcactatagggctcgagcgcccgcccgggcaggtataatattagacttgtactcaatgacaagcgccatctatgagtttcatcatgcctatatataaacacatgaacctgtcattgttcatttatgcattattgttgtattagctgaaaaatttctggcaaatgacgcgattatattctgtgttctttcttttgttggctcttgtagttgaaccgggtgttagagcctggagcaaagaaggccatgtcatgacatgtcaaattgcgcaggatctgttggagccagaagcagcacatgctgtaaagatgctgttaccggactatgctaatggcaacttatcgtcgctgtgtgtgtggcctgatcaaattcgacactggtacaagtacaggtggactagctctctccatttcatcgatacacctgatcaagcctgttcatttgattaccagagagactgtcatgatccacatggagggaaggacatgtgtgttgctggagccattcaaaatttcacatctcagcttggacatttccgccatggaacatctgatcgtcgatataatatgacagaggctttgttatttttatcccacttcatgggagatattcatcagcctatgcatgttggatttacaagtgatatgggaggaaacagtatagatttgcgctggtttcgccacaaatccaacctgcaccatgtttgggatagagagattattcttacagctgcagcagattaccatggtaaggatatgcactctctcctacaagacatacagaggaactttacagagggtagttggttgcaagatgttgaatcctggaaggaatgtgatgatatctctacttgcgccaataagtatgctaaggagagtataaaactagcctgtaactggggttacaaagatgttgaatctggcgaaactctgtcagataaatacttcaacacaagaatgccaattgtcatgaaacggatagctcagggtggaatccgtttatccatgattttgaaccgagttcttggaagctccgcagatcattctttggcatgaatttagatactgatattcgcatttctcatgacacccttctcttatgcaatttgcagatcagctgtgattcactaattgaa

SEQ ID NO: 4 - protein, 296 aa, Apium sp.
MTRLYSVFFLLLALVVEPGVRAWSKEGHVMTCQIAQDLLEPEAAHAVKMLLPDYANGNLSSLCVWPDQIRHWYKYRWTSSLHFIDTPDQACSFDYQRDCHDPHGGKDMCVAGAIQNFTSQLGHFRHGTSDRRYNMTEALLFLSHFMGDIHQPMHVGFTSDMGGNSIDLRWFRHKSNLHHVWDREIILTAAADYHGKDMHSLLQDIQRNFTEGSWLQDVESWKECDDISTCANKYAKESIKLACNWGYKDVESGETLSDKYFNTRMPIVMKRIAQGGIRLSMILNRVLGSSADHSLA

SEQ ID NO: 5 - DNA, 933 bp, Apium sp.
atgggtatgttgacttatactggaatttattttctgctattacttccaagtgttttctgttggggaaaacaaggacattttgcaatttgtaaaattgcccaggggttccttagtaaagatgcactgactgcagtgaaagcattgctcccagaatatgcagatggtgatctagcagctgtttgctcctgggctgacgaggttcgatttcatatgcgttggagtagcccattacattatgtggacacgcctgatttcaggtgtaactataaatactgtagagattgccatgattctgttggacggaaagaccggtgtgttactggagcaattcacaactacacagagcaacttctattgggtgttcatgacttgaattcaaaaatgaataacaacttgacggaggcacttatgttcttatcacatttcgttggtgatgtccatcagcctctacatgttggcttccttggcgatgaaggaggaaacacaatcaccgtccgctggtatcggaggaaaaccaatttgcatcatgtatgggacacaatgatgattgaatcctccttgaagacattctacaattcagatctttctagcttaatacaagctattcagagcaatattacaggtgtctggcttaccgacagcttatcttggagcaattgcactgctgatcatgtggtttgtccagacccgtatgcttctgaaagcattgagttggcctgcaagtttgcctacagaaatgccacacctgggaccactttaggagatgagtacttcctctctcggttgcctgttgcggagaagaggttggctcaggctggggtccgtttggctgctactcttaaccgaatcttcacttcaaaccccagcgatctcacaagattgaatatgcataatggtggacatagaagcagtaacaatattgaaatagtgtaa

SEQ ID NO: 6 - protein, 310 aa, Apium sp.
MGMLTYTGIYFLLLLPSVFCWGKQGHFAICKIAQGFLSKDALTAVKALLPEYADGDLAAVCSWADEVRFHMRWSSPLHYVDTPDFRCNYKYCRDCHDSVGRKDRCVTGAIHNYTEQLLLGVHDLNSKMNNNLTEALMFLSHFVGDVHQPLHVGFLGDEGGNTITVRWYRRKTNLHHVWDTMMIESSLKTFYNSDLSSLIQAIQSNITGVWLTDSLSWSNCTADHVVCPDPYASESIELACKFAYRNATPGTTLGDEYFLSRLPVAEKRLAQAGVRLAATLNRIFTSNPSDLTRLNMHNGGHRSSNNIEIV

SEQ ID NO: 7 - DNA, 873 bp, Apium sp.
tggggaaaacaaggacattttgcaatttgtaaaattgcccaggggttccttagtaaagatgcactgactgcagtgaaagcattgctcccagaatatgcagatggtgatctagcagctgtttgctcctgggctgacgaggttcgatttcatatgcgttggagtagcccattacattatgtggacacgcctgatttcaggtgtaactataaatactgtagagattgccatgattctgttggacggaaagaccggtgtgttactggagcaattcacaactacacagagcaacttctattgggtgttcatgacttgaattcaaaaatgaataacaacttgacggaggcacttatgttcttatcacatttcgttggtgatgtccatcagcctctacatgttggcttccttggcgatgaaggaggaaacacaatcaccgtccgctggtatcggaggaaaaccaatttgcatcatgtatgggacacaatgatgattgaatcctccttgaagacattctacaattcagatctttctagcttaatacaagctattcagagcaatattacaggtgtctggcttaccgacagcttatcttggagcaattgcactgctgatcatgtggtttgtccagacccgtatgcttctgaaagcattgagttggcctgcaagtttgcctacagaaatgccacacctgggaccactttaggagatgagtacttcctctctcggttgcctgttgcggagaagaggttggctcaggctggggtccgtttggctgctactcttaaccgaatcttcacttcaaaccccagcgatctcacaagattgaatatgcataatggtggacatagaagcagtaacaatattgaaatagtgtaa

SEQ ID NO: 8 - protein, 290 aa, Apium sp.
WGKQGHFAICKIAQGFLSKDALTAVKALLPEYADGDLAAVCSWADEVRFHMRWSSPLHYVDTPDFRCNYKYCRDCHDSVGRKDRCVTGAIHNYTEQLLLGVHDLNSKMNNNLTEALMFLSHFVGDVHQPLHVGFLGDEGGNTITVRWYRRKTNLHHVWDTMMIESSLKTFYNSDLSSLIQAIQSNITGVWLTDSLSWSNCTADHVVCPDPYASESIELACKFAYRNATPGTTLGDEYFLSRLPVAEKRLAQAGVRLAATLNRIFTSNPSDLTRLNMHNGGHRSSNNIEIV

SEQ ID NO: 9 - DNA, 921 bp, Mimulus guttatus
atgcagatgtcgatttcacgaggaatttttgtttcttattttgctttatttctttgtgtttgtgttgtttatgaaccttgtgtccaggcatggagtaaagaaggtcattccatgacatgcaaaattgctcaggatttgctgggaccagaggcgaagcatgctgtccaaatgctgttacctgaaaatgttaatggtgatttatcggcacttagcgtgtggcctgaccaagtaagacactggtataagtaccgttggacgagccctcttcacttcatagacacaccagatcaagcctgtaatttcaattatcagagggattgccatgatccacatggtgttaagggtatgtgtgtagcgggggcaattcagaacttcaccaatcagctttcgcattatcggcacggaacctctgatcgacgctataatatgacagaggccttgttgttcttggcacacttcatgggagatattcatcagccactgcatgttggattcacgagtgacgaaggaggaaacactatagacttgcgctggttcagacacaagtcaaatctgcaccatgtatgggacagagagataattcttacagctgcagcagattactacggaaaggacattgacctcctgcaagaagacattaagggaaacttcactgatggaatctggtctggtgatcttgcctcttggagggaatgcagtgatatattttcttgtgtcaacaagtatgctgctgagagtataaacatggcctgcaaatggggttacaaagatgttaaatcaggggacactctttcagatgattactttaattcaagattgccgattgttatgaaacgcatagctcagggtggagtccgtttagctatgattttgaaccgggttttcggtgatagcaaagaggattccttaattgctacttaa

SEQ ID NO: 10 - protein, 306 aa, Mimulus guttatus
MQMSISRGIFVSYFALFLCVCVVYEPCVQAWSKEGHSMTCKIAQDLLGPEAKHAVQMLLPENVNGDLSALSVWPDQVRHWYKYRWTSPLHFIDTPDQACNFNYQRDCHDPHGVKGMCVAGAIQNFTNQLSHYRHGTSDRRYNMTEALLFLAHFMGDIHQPLHVGFTSDEGGNTIDLRWFRHKSNLHHVWDREIILTAAADYYGKDIDLLQEDIKGNFTDGIWSGDLASWRECSDIFSCVNKYAAESINMACKWGYKDVKSGDTLSDDYFNSRLPIVMKRIAQGGVRLAMILNRVFGDSKEDSLIAT

SEQ ID NO: 11 - protein, 308 aa, Artificial Sequence
  Synthetic construct: Insect Cell Expression
MKFLVNVALVFMVVYISYIYAWSKEGHSMTCKIAQDLLGPEAKHAVQMLLPENVNGDLSALSVWPDQVRHWYKYRWTSPLHFIDTPDQACNFNYQRDCHDPHGVKGMCVAGAIQNFTNQLSHYRHGTSDRRYNMTEALLFLAHFMGDIHQPLHVGFTSDEGGNTIDLRWFRHKSNLHHVWDREIILTAAADYYGKDIDLLQEDIKGNFTDGIWSGDLASWRECSDIFSCVNKYAAESINMACKWGYKDVKSGDTLSDDYFNSRLPIVMKRIAQGGVRLAMILNRVFGDSKEDSLIATGSHHHHHHHHG

SEQ ID NO: 12 - DNA, 909 bp, Solanum tuberosum
atgttgaggttaacttcattaagcattattttctttctctgtcttgcttttatcaaccatcatggtgctgaagcatggagcaaagaggggcatatgatgacatgtcgcatcgcgcagggcttgttgaatgatgaggcagctcatgcagtcaagatgttgttgccggaatatgttaacggcgacttatcggccctctgtgtgtggccggatcaagtccggcactggtataagtataaatggacaagccctctacacttcattgatacaccagataaagcttgcaactttgattatgaaagggactgtcatgatcaacatggagtgaaggatatgtgtgttgctggtgcaattcagaactttactactcaactctctcattacagagagggaacttctgatcgtcgatataatatgacagaggccttgctgttcttgtcacattttatgggagatatccatcaaccaatgcatgttggctttacaagtgatgctggaggaaatagtattgatttacgctggtttaggcataaatcgaacttgcaccatgtgtgggatagggagataattctaacagctgctaaagactactatgcaaaggatgtaaacctccttgaagaagacattgaaggaaacttcactgacggaatttggtctgatgatcttgcttcttggagagaatgtggcaatgtcttttcttgtgtaaacaagtttgcaacggaaagtataaatatagcatgcaaatggggatacaaaagtgttgaagctggtgaaactttatcagatgattatttcaattcaagacttccaatagtgatgaaacgagtagcacaaggtggaatacgattagccatgcttttaaacaacgtttttggagtttctcaacaagaagattcagttgctgcaacttaa

SEQ ID NO: 13 - protein, 302 aa, Solanum tuberosum
MLRLTSLSIIFFLCLAFINHHGAEAWSKEGHMMTCRIAQGLLNDEAAHAVKMLLPEYVNGDLSALCVWPDQVRHWYKYKWTSPLHFIDTPDKACNFDYERDCHDQHGVKDMCVAGAIQNFTTQLSHYREGTSDRRYNMTEALLFLSHFMGDIHQPMHVGFTSDAGGNSIDLRWFRHKSNLHHVWDREIILTAAKDYYAKDVNLLEEDIEGNFTDGIWSDDLASWRECGNVFSCVNKFATESINIACKWGYKSVEAGETLSDDYFNSRLPIVMKRVAQGGIRLAMLLNNVFGVSQQEDSVAAT

SEQ ID NO: 14 - protein, 276 aa, Mimulus guttatus
WSKEGHSMTCKIAQDLLGPEAKHAVQMLLPENVNGDLSALSVWPDQVRHWYKYRWTSPLHFIDTPDQACNFNYQRDCHDPHGVKGMCVAGAIQNFTNQLSHYRHGTSDRRYNMTEALLFLAHFMGDIHQPLHVGFTSDEGGNTIDLRWFRHKSNLHHVWDREIILTAAADYYGKDIDLLQEDIKGNFTDGIWSGDLASWRECSDIFSCVNKYAAESINMACKWGYKDVKSGDTLSDDYFNSRLPIVMKRIAQGGVRLAMILNRVFGDSKEDSLIAT

SEQ ID NO: 15 - DNA, 831 bp, Vitis vinifera
atgtggggaaaggaaggacactatgcagtttgtaaaatagctgaggggttcctttctgaagatgcattaggagcagtgaaaggattgcttccagattatgctgatggtgatctggctgccgtttgctcctgggctgatgagattcgtcacaacttccattggcgatggagtggccctttacattatgtagatacaccagattacaggtgtaattatgaatactgcagagactgccatgacttcagaggacacaaagatatatgtgtaactggagcaatttacaactacacaaagcaactcacttctggttatcacaattcaggttcagaaataagatacaatttgacagaggccctcatgttcttatcagattttattggggatgtccatcagcccctacatgttggttttactggagatgaaggtgggaacacaataatagtccgttggtaccggaggaagactaatttgcatcatatatgggatgacatgatcattgattccgccttgaagacatattacaattcagatattgcaatcatgatacaagccattcaaagaaatattacaggtgactggtcctttgatatctcatcatggaaaaattgtgcatctgatgatacggcttgtccaaacctgtatgcgtctgaaggcattagtttagcttgcaagtttgcttacagaaatgccacaccaggaagcactctaggagatgattacttcctgtctcggctaccaattgtggagaagaggctagccccgagtgggatccgcctggctgccacccttaaccgtatctttgcttctcaaggcaagagagctaaagcatga

SEQ ID NO: 16 - protein, 276 aa, Vitis vinifera
MWGKEGHYAVCKIAEGFLSEDALGAVKGLLPDYADGDLAAVCSWADEIRHNFHWRWSGPLHYVDTPDYRCNYEYCRDCHDFRGHKDICVTGAIYNYTKQLTSGYHNSGSEIRYNLTEALMFLSDFIGDVHQPLHVGFTGDEGGNTIIVRWYRRKTNLHHIWDDMIIDSALKTYYNSDIAIMIQAIQRNITGDWSFDISSWKNCASDDTACPNLYASEGISLACKFAYRNATPGSTLGDDYFLSRLPIVEKRLAPSGIRLAATLNRIFASQGKRAKA

SEQ ID NO: 17 - protein, 331 aa, Artificial Sequence
  Synthetic construct: Insect Cell Expression
MKFLVNVALVFMVVYISYIYAWGKEGHYAVCKIAEGFLSEDALGAVKALLPDYAEGDLAAVCSWADEIRHNFHWRWSGPLHYVDTPDYRCNYEYCRDCHDFRGHKDICVTGAIYNYTKQLTSGYHNSGSEIRYNLTEALMFLSHFIGDVHQPLHVGFTGDEGGNTIIVRWYRRKTNLHHIWDNMIIDSALKTYYNSDLAIMIQAIQRNITGDWSFDISSWKNCASDDTACPNLYASESISLACKFAYRNATPGSTLGDDYFLSRLPIVEKRLAQGGIRLAATLNRIFASQPKISLKHEDKRVEKTTPVDYIEWSPLQQFSGSHHHHHHHHG

SEQ ID NO: 18 - DNA, 840 bp, Artificial Sequence
  Synthetic construct: Chocolate pots
atgacttggggattttgggcacatcggcaaatacatcgccaagccgtttatcttatgccttcgcccgtggcagagttctttcgcgcaaatgttcaagaacttgtcgaccgctcggttgaagccgatgaacgccgacgcatagaccccaacgaagctccgcaacacttcattgatttagaccgctacggtgcctatccttttgaacaacttccgagagattatgaaaaagccgttgagaaattcggctatgagcggctgaaagaaaatggacttgtgccgtggcgcattgccgcctttgccgatagcctcaccaacgcatttcgggagcagaaccgcgaaaaaattttatacttcgccgcaaatttagggcattatgtcgccgatgctaacgtgccacttcatgccaccgaaaactacgacggacaactcacagggcaaaaaggattgcacgcacgttgggaaactatttatcctcaaaagtttatgctcccacgagaaaccacctatctcgaaaacgggagcatctttatcattgacaacatcaccgaagaagccttcaactggtcattagaaagttatgtattgagccaacaagttttggcgattgataagcaaattcaatcggaattgtcagaagaagaattgtatgagttaaattcatcagacgcgccgccatttcgtcgcgatttttcacaacgctattatgaaaaactcaaagaaaaattgaatcaaatggttgaaaaatgctttgagttaagcgtcattagggtagcgtcagtttggtatttttcttggttaaaagcagaaaaaccgaatttatttaacttattaaaaaattga

SEQ ID NO: 19 - protein, 279 aa, Artificial Sequence
  Synthetic construct: Chocolate pots
MTWGFWAHRQIHRQAVYLMPSPVAEFFRANVQELVDRSVEADERRRIDPNEAPQHFIDLDRYGAYPFEQLPRDYEKAVEKFGYERLKENGLVPWRIAAFADSLTNAFREQNREKILYFAANLGHYVADANVPLHATENYDGQLTGQKGLHARWETIYPQKFMLPRETTYLENGSIFIIDNITEEAFNWSLESYVLSQQVLAIDKQIQSELSEEELYELNSSDAPPFRRDFSQRYYEKLKEKLNQMVEKCFELSVIRVASVWYFSWLKAEKPNLFNLLKN

SEQ ID NO: 20 - DNA, 807 bp, Unknown
  Obsidian pool
atgttttgggcacatcaaaaagtcaacgagcatgccattgatttattacccgagccactccgcagtttttatgaacaaaataaggaatacatagttaaggagtcggtcgcccctgatctcaggcgtgcagaaaacaaggaagaaggttattatcactatatggatctcgataaatatggtgaatatccgttcaagaatttgccagaaaactacgacgacgcagtaaaaaggtttggttacgatactgttctcaagaacggaattgtgccgtggaaggtaaaatggttgacagacagtttgagtcaagctatggagagaaaggatgtgccacaggtcttaagactttcagccgaccttggtcattatgttgctgacatgcatgttccatttcattcgacagaaaattatgatggacagctgacaggcaacataggaatacacttcagatgggaaagcggcattccagaacattttggaacaaattacaactatgagggaatagagcccgctgtttacttcaagcatcctgataaaaaggcatttgagatactgactatgagttacaagttgattctaccttctctcaaggctgatagtcttgcaaaagttggattgaatggaaagagactttataaagttgagagagaagacggtaaaaaagtttacgtttattcaaacgagtattatgagaagttcaacaaaaaccttggtggtattgtagaatcgcagatgaggctggcaatccatgatgttgcaagctactggtatactgcatgggtaaatgccggtaaaccaaagttttggtaa

SEQ ID NO: 21 - protein, 268 aa, Unknown
  Obsidian pool
MFWAHQKVNEHAIDLLPEPLRSFYEQNKEYIVKESVAPDLRRAENKEEGYYHYMDLDKYGEYPFKNLPENYDDAVKRFGYDTVLKNGIVPWKVKWLTDSLSQAMERKDVPQVLRLSADLGHYVADMHVPFHSTENYDGQLTGNIGIHFRWESGIPEHFGTNYNYEGIEPAVYFKHPDKKAFEILTMSYKLILPSLKADSLAKVGLNGKRLYKVEREDGKKVYVYSNEYYEKFNKNLGGIVESQMRLAIHDVASYWYTAWVNAGKPKFW

SEQ ID NO: 22 - DNA, 972 bp, Vitis vinifera
atggcttggtctggggtcttgttgattgtgagggcacttgttcttctgcaattgattcctggaattctgagttggggaaaggaaggacactatgcagtttgtaaaatagctgaggggttcctttctgaagatgcattaggagcagtgaaagcattgcttccagattatgctgaaggtgatctggctgcggtttgctcctgggctgatgagattcgtcacaacttccattggcgatggagtggccctttacattatgtagatacgccagattacaggtgtaactatgaatactgcagagactgccatgacttcagaggacacaaagatatatgtgtaactggagcaatttacaattacacaaagcaactcacttctggttatcacaattcaggttcagaaataagatacaatttgacagaggcactcatgttcttatcacattttattggggatgtccatcagcccctacatgttggttttactggagatgaaggtgggaacacaataatagtccgttggtaccggaggaagactaatttgcatcatatatgggataacatgatcattgattccgccctgaagacatattacaattcagatcttgcaatcatgatacaagccattcaaagaaatattacgggtgattggtcctttgatatctcatcatggaaaaattgtgcatctgatgatacggcttgtccaaacctgtatgcttctgaaagcattagtttagcttgcaagtttgcttacagaaatgccacaccaggaagcactctaggagatgattacttcctgtctcggctaccaattgtggagaagaggctagcccaaggtgggatccgcctggctgccacccttaaccgtatctttgcttctcaaccaaaaatctctctcaagcatgaagataaaagggtagagaaaacaactccagtggattatatagagtggagcccactgcaacaattttcataa

SEQ ID NO: 23 - protein, 323 aa, Vitis vinifera
MAWSGVLLIVRALVLLQLIPGILSWGKEGHYAVCKIAEGFLSEDALGAVKALLPDYAEGDLAAVCSWADEIRHNFHWRWSGPLHYVDTPDYRCNYEYCRDCHDFRGHKDICVTGAIYNYTKQLTSGYHNSGSEIRYNLTEALMFLSHFIGDVHQPLHVGFTGDEGGNTIIVRWYRRKTNLHHIWDNMIIDSALKTYYNSDLAIMIQAIQRNITGDWSFDISSWKNCASDDTACPNLYASESISLACKFAYRNATPGSTLGDDYFLSRLPIVEKRLAQGGIRLAATLNRIFASQPKISLKHEDKRVEKTTPVDYIEWSPLQQFS

SEQ ID NO: 24 - DNA, 891 bp, Solanum sp.
atgggtgggtttgagctcaaatggtttgtaggagtagctgttgttctgatgatggttcaaaatattcttggttgggggaaagagggacactatattatctgcaaaattgctgaggaatatctaacagaagatgctttagctgcagtcaaagcattactcccagatcaagccgaaggtgatcttgcagctgtctgctcctggcctgatgaggttcggcgccactaccactaccgctggagctctccattacattatgtagatacacctgatttcttgtgcaattacaaatattgccgagactgccatgacgggcatgggctcaaggacaggtgtgttacgggagcaatatacaactactcaatgcaactttcgcagggatattatgatttgaattcagaaaaatacaacttgactgaagcacttatgttcttgtctcattttgttggtgacgtacatcagcctctccatgttggtttcactggagatcttggtggaaacagtataattgttcgttggtacaggaggaagactaatttgcaccatgtatgggataacatgattattgaatctgcgttgaagacatactacaaatctgatataatgttaatgacacaagttcttctgaaaaacatcactcatgaatggtccgatgatgttccatcttgggaagattgcaaggagatggtttgtcctgacccatatgcttctgaaagtatccgtttggcctgcaaatttgcctacagaaatgcaaccccgggaagcactttaacagacgattacttcctctctcgtcttcctgttgtggagaagaggttggcacaaggtggggtccgcttggccgaagttctcaacagaattttcactaaaaaaccatcagatgctgcacaatga

SEQ ID NO: 25 - protein, 296 aa, Solanum tuberosum
MGGFELKWFVGVAVVLMMVQNILGWGKEGHYIICKIAEEYLTEDALAAVKALLPDQAEGDLAAVCSWPDEVRRHYHYRWSSPLHYVDTPDFLCNYKYCRDCHDGHGLKDRCVTGAIYNYSMQLSQGYYDLNSEKYNLTEALMFLSHFVGDVHQPLHVGFTGDLGGNSIIVRWYRRKTNLHHVWDNMIIESALKTYYKSDIMLMTQVLLKNITHEWSDDVPSWEDCKEMVCPDPYASESIRLACKFAYRNATPGSTLTDDYFLSRLPVVEKRLAQGGVRLAEVLNRIFTKKPSDAAQ

SEQ ID NO: 26 - DNA, 885 bp, Medicago sp.
atgatcacgctcttagttccgttgctgctatcactcgcgttgccaaatgttctggcttggggaaaagatggtcactatgcaatttgtaaaatttcacaggagtatcttagtgaagatgctctatttgcagtcaaacaattacttccagattctgctcaagctgatcttgcttcagtttgctcttggcctgatgagattcgccataattaccattatcgttggagtagtcctttacattatattgatacaccagatttcaaatgtaactatcaatattgcagagactgtcatgattcttatggacataagcatagatgcgttactggagcaatatacaattatacaatgcaattaaaattagctaacgccgatgcttcatctgaattaaaatataacttgacagaggcacttatgttcttgtcacattttgttggagatgttcatcagcccctacatgttggttttactggagacctaggtggaaactcaataacagttcgttggtacaggaggaaaacaaatcttcatcacgtatgggataacatgattattgagtctgctctgaaaaagttctatggttcagatctttcaactatgatacaggctattcaaaggaatattagtgatatttggtcaaatgatgtatctatttgggaacattgtgcacacaaccacacagcatgtccagaccggtatgcttctgagagtattagcttggcatgcaagtttgcgtataagaatgctacaccgggaagcactttggaagatgactacttcctttctcggttgcctattgtggagaaaaggctggctcaaggtggtgtgcgacttgcagctatcctcaaccacattttcactccgaagaccagaatagctcaagcttaa

SEQ ID NO: 27 - protein, 294 aa, Medicago sp.
MITLLVPLLLSLALPNVLAWGKDGHYAICKISQEYLSEDALFAVKQLLPDSAQADLASVCSWPDEIRHNYHYRWSSPLHYIDTPDFKCNYQYCRDCHDSYGHKHRCVTGAIYNYTMQLKLANADASSELKYNLTEALMFLSHFVGDVHQPLHVGFTGDLGGNSITVRWYRRKTNLHHVWDNMIIESALKKFYGSDLSTMIQAIQRNISDIWSNDVSIWEHCAHNHTACPDRYASESISLACKFAYKNATPGSTLEDDYFLSRLPIVEKRLAQGGVRLAAILNHIFTPKTRIAQA

SEQ ID NO: 28 - protein, 271 aa, Artificial Sequence
  Synthetic construct
WGKEGHYAVCKIAEGFLSEDALGAVKGLLPDYADGDLAAVCSWADEIRHNFHWRWSGPLHYVDTPDYRCNYEYCRDCHDFRGHKDICVTGAIYNYTKQLTSGYHNSGSEIRYNLTEALMFLSDFIGDVHQPLHVGFTGDEGGNTIIVRWYRRKTNLHHIWDDMIIDSALKTYYNSDIAIMIQAIQRNITGDWSFDISSWKNCASDDTACPNLYASEGISLACKFAYRNATPGSTLGDDYFLSRLPIVEKRLAPSGIRLAATLNRIFASQGK

SEQ ID NO: 29 - protein, 271 aa, Vitis vinifera
WGKEGHYAVCKIAEGFLSEDALGAVKALLPDYAEGDLAAVCSWADEIRHNFHWRWSGPLHYVDTPDYRCNYEYCRDCHDFRGHKDICVTGAIYNYTKQLTSGYHNSGSEIRYNLTEALMFLSHFIGDVHQPLHVGFTGDEGGNTIIVRWYRRKTNLHHIWDNMIIDSALKTYYNSDLAIMIQAIQRNITGDWSFDISSWKNCASDDTACPNLYASESISLACKFAYRNATPGSTLGDDYFLSRLPIVEKRLAQGGIRLAATLNRIFASQPK

SEQ ID NO: 30 - DNA, 828 bp, Artificial Sequence
  Synthetic construct: Codon Optimized Mature Core Mimulus DNA Encodes SEQ ID NO:14
tggagtaaggagggacatagcatgacatgtaagatagcccaggacttgttgggtcccgaagccaaacacgccgtgcaaatgttgttgcctgaaaatgtgaacggcgacctaagcgccttgtcggtgtggccggaccaagtgagacactggtacaaatacagatggacctcccctttgcacttcattgacacccccgatcaggcttgcaactttaactaccagagagactgccatgacccgcacggtgtaaaaggcatgtgcgttgccggtgccattcaaaatttcacgaaccaattgtcgcactacagacacggcacgtcggacagacgttacaacatgacggaggccttgttgtttttggcccactttatgggcgatattcatcagccgttgcacgtgggcttcacgtcagacgaaggcggcaacacgattgacttgagatggtttcgccacaagagcaacttgcatcacgtatgggatcgagaaattatcctaactgccgctgcggactactacggaaaggacatcgacctactccaggaggatatcaaaggcaattttactgacggcatctggtcgggcgatttggcctcgtggagagaatgttcggacattttttcgtgtgtgaacaagtacgctgccgaatccataaacatggcttgtaaatggggctacaaggatgtgaaatcgggtgacacgctctcggacgactatttcaacagtcgtctcccgatcgtaatgaaaagaatcgctcaaggaggcgttcgcttagcaatgattctcaacagagtattcggtgatagcaaagaggacagcttgattgccacg

SEQ ID NO: 31 - DNA, 933 bp, Artificial Sequence
  Synthetic construct: Blue Sky Report Mimulus DNA Encodes SEQ ID NO:11
accatgaagttcttggtcaacgtagcactggtttttatggtagtctatatcagctacatttacgcgtggagtaaggagggacatagcatgacatgtaagatagcccaggacttgttgggtcccgaagccaaacacgccgtgcaaatgttgttgcctgaaaatgtgaacggcgacctaagcgccttgtcggtgtggccggaccaagtgagacactggtacaaatacagatggacctcccctttgcacttcattgacacccccgatcaggcttgcaactttaactaccagagagactgccatgacccgcacggtgtaaaaggcatgtgcgttgccggtgccattcaaaatttcacgaaccaattgtcgcactacagacacggcacgtcggacagacgttacaacatgacggaggccttgttgtttttggcccactttatgggcgatattcatcagccgttgcacgtgggcttcacgtcagacgaaggcggcaacacgattgacttgagatggtttcgccacaagagcaacttgcatcacgtatgggatcgagaaattatcctaactgccgctgcggactactacggaaaggacatcgacctactccaggaggatatcaaaggcaattttactgacggcatctggtcgggcgatttggcctcgtggagagaatgttcggacattttttcgtgtgtgaacaagtacgctgccgaatccataaacatggcttgtaaatggggctacaaggatgtgaaatcgggtgacacgctctcggacgactatttcaacagtcgtctcccgatcgtaatgaaaagaatcgctcaaggaggcgttcgcttagcaatgattctcaacagagtattcggtgatagcaaagaggacagcttgattgccacgggctcgcaccatcaccaccatcaccaccacggttgataa

SEQ ID NO: 32 - DNA, 897 bp, Artificial Sequence
  Synthetic construct: Codon Optimized Vitis DNA Encodes Residues XXX YYY of SEQ ID NO:23
tggggcaaagaaggccactacgccgtgtgtaagattgcggagggctttttgtcggaagacgcattgggagcggtcaaagccttgttgccggactacgcggaaggcgacttggcagccgtatgtagctgggccgacgagatcagacacaactttcactggagatggtcgggcccactgcattacgtcgacacgccggattacagatgcaactacgagtactgccgcgactgtcacgacttcagaggccacaaagacatttgcgtcacgggcgcgatatacaactacacgaaacaattgacgtcgggctaccacaacagtggctccgagattcgatacaacctcacggaggccttgatgttcctctcgcatttcattggcgacgtgcaccaaccgctgcatgtgggctttacgggcgatgaaggcggaaatacgatcattgtccgttggtaccgcagaaagaccaacctccaccacatatgggacaacatgatcatcgactcggcgttgaagacctactacaacagcgacctggccataatgatccaggcgattcaaagaaacatcaccggcgattggtcctttgacatcagcagctggaagaactgtgccagtgacgacactgcttgtccgaacctatacgcgtcggagagcatctcgttggcctgtaaatttgcctacagaaatgccacccccggttcgacgctgggcgacgactacttcttgtcgcgattgccgattgttgaaaaacgcctcgcccaaggcggtattagattggccgccaccttgaaccgtatttttgcctcgcaaccgaaaatctcgctgaaacacgaagacaagagagtcgagaagacgacgccggtagactacatcgagtggtcgccattgcaacagttcagc

SEQ ID NO: 33 - DNA, 1002 bp, Artificial Sequence
  Synthetic construct: Blue Sky Report Vitis DNA Encodes SEQ ID NO:17
accatgaagttcttggtgaacgtggcgctggtgttcatggtcgtgtacatctcctacatttacgcgtggggcaaagaaggccactacgccgtgtgtaagattgcggagggctttttgtcggaagacgcattgggagcggtcaaagccttgttgccggactacgcggaaggcgacttggcagccgtatgtagctgggccgacgagatcagacacaactttcactggagatggtcgggcccactgcattacgtcgacacgccggattacagatgcaactacgagtactgccgcgactgtcacgacttcagaggccacaaagacatttgcgtcacgggcgcgatatacaactacacgaaacaattgacgtcgggctaccacaacagtggctccgagattcgatacaacctcacggaggccttgatgttcctctcgcatttcattggcgacgtgcaccaaccgctgcatgtgggctttacgggcgatgaaggcggaaatacgatcattgtccgttggtaccgcagaaagaccaacctccaccacatatgggacaacatgatcatcgactcggcgttgaagacctactacaacagcgacctggccataatgatccaggcgattcaaagaaacatcaccggcgattggtcctttgacatcagcagctggaagaactgtgccagtgacgacactgcttgtccgaacctatacgcgtcggagagcatctcgttggcctgtaaatttgcctacagaaatgccacccccggttcgacgctgggcgacgactacttcttgtcgcgattgccgattgttgaaaaacgcctcgcccaaggcggtattagattggccgccaccttgaaccgtatttttgcctcgcaaccgaaaatctcgctgaaacacgaagacaagagagtcgagaagacgacgccggtagactacatcgagtggtcgccattgcaacagttcagcggaagccaccaccatcaccaccatcatcacggctgataa